European Patent Application EP 4 545 637 A1, published April 30, 2025. Title: N-terminal and/or C-terminal Cleaved Soluble PH20 polypeptide and Use Thereof. Applicant: Alteogen Inc. The sequence listing filed with the application follows.

SEQUENCE LISTING (10 sequences)

SEQ ID NO: 1 - protein, 509 aa, synthetic construct
  REGION 1..509: note = Synthetic Sequence
MGVLKFKHIFFRSFVKSSGVSQIVFTFLLIPCCLTLNFRAPPVIPNVPFLWAWNAPSEFCLGKFDEPLDMSLFSFIGSPRINATGQGVTIFYVDRLGYYPYIDSITGVTVNGGIPQKISLQDHLDKAKKDITFYMPVDNLGMAVIDWEEWRPTWARNWKPKDVYKNRSIELVQQQNVQLSLTEATEKAKQEFEKAGKDFLVETIKLGKLLRPNHLWGYYLFPDCYNHHYKKPGYNGSCFNVEIKRNDDLSWLWNESTALYPSIYLNTQQSPVAATLYVRNRVREAIRVSKIPDAKSPLPVFAYTRIVFTDQVLKFLSQDELVYTFGETVALGASGIVIWGTLSIMRSMKSCLLLDNYMETILNPYIINVTLAAKMCSQVLCQEQGVCIRKNWNSSDYLHLNPDNFAIQLEKGGKFTVRGKPTLEDLEQFSEKFYCSCYSTLSCKEKADVKDTDAVDVCIADGVCIDAFLKPPMETEEPQIFYNASPSTLSATMFIVSILFLIISSVASL

SEQ ID NO: 2 - protein, 510 aa, synthetic construct
  REGION 1..510: note = Synthetic Sequence
MGVIKFKHIFFRSFVKSSGVSQIVFTFLLIPCCLTLNFRAPPIIPNVPFLWAWNAPSEFCLGKFDEPLDMSLFSLIGSPRINVTGQGVTIFYVDRLGYYPYIDITTGVTVHGGIPQKVSLQDHLDKAKQDIIFYMPVDNLGMAVIDWEEWRPTWARNWKPKDVYKNRSIELVQQQNVQLSLPEATDKAKQEFEKAGKDFMLETIKLGKSLRPNHLWGYYLFPDCYNHHYKKPGYNGSCFDVEIKRNDDLSWLWNESTALYPSIYLNTQQSPVAATLYVRNRVQEAIRVSKIPDAKNPLPVFVYARLVFTDQVLKFLSRDELVYTLGETVALGASGIVIWGSLSIMRSMKSCLLLDNYMETILNPYIINVTLAAKMCSQVLCQEQGVCIRKDWNSSDYLHLNPDNFAIQMEKGGKFTVRGKPTLEDLEEFSEKFYCSCYTTLSCKEKADVKDTDAVDVCIADGVCIDASLKPPVETEGSPPIFYNTSPSTLSTTMFIVSILFLIISSVVSL

SEQ ID NO: 3 - protein, 509 aa, synthetic construct
  REGION 1..509: note = Synthetic Sequence
MGVLKFKHIFFRSFVKSSGVSQIVFTFLLIPCCLTLNFRAPPVIPNVPFLWAWNAPSEFCLGKFDEPLDMSLFSFIGSPRINVTGQDVTIFYVDRLGYYPYIDSITGVTVNGGIPQKISLQDHLDKAKKDITFYMPVDNLGMAVIDWEEWRPTWARNWKPKDVYKNRSIELVQQQNVQLSLTEATEKAKQEFEKAGKDFLVETIKLGKLLRPNHLWGYYLFPDCYNHHYKKPGYNGSCFNVEIKRNDDLSWLWNESTALYPSIYLNTQQSPVAATLYVRNRVQEAIRVSKIPDAKSPLPVFVYTRIVFTDQVLKFLSQDELVYTFGETVALGASGIVIWGTLSIMRSMKSCLLLDNYMETILNPYIINVTLAAKMCSQVLCQEQGVCIRKNWNSSDYLHLNPDNFAIQLEKGGKFTVRGKPTLEDLEQFSEKFYCSCYSTLSCKEKADVKDTDAVDVCIADGVCIDAFLKPPMETEESQIFYNASPSTLSATMFIVSILFLIISSVASL

SEQ ID NO: 4 - protein, 509 aa, synthetic construct
  REGION 1..509: note = Synthetic Sequence
MGVLKFKHIFFGSFVKSSGVSQIVFTFLLIPCCLTLNFRAPPVIPNVPFLWAWNAPSEFCLGKFDEPLDMSLFSFIGSPRINVTGQDVTIFYVDRLGYYPYIDSITGVTVNGGIPQKISLQDHLDKAKKDITFYMPVDNLGMAVIDWEEWRPTWARNWKPKDIYKNRSIELVQQQNVQLNLTEATEKAKQEFEKAGKDFLVETIKLGKLLRPNHLWGYYLFPDCYNHHYKKPGYNGSCFNVEIKRNDDLSWLWNESTALYPSIYLNTQQSPVAATLYVRNRVREAIRVSKIPDAKSPLPVFVYTRIVFTDQVLKFLSQDELVYTFGETVALGASGIVIWGTLSIMRSMKSCLLLDNYMETILNPYIINVTLAAKMCSQVLCQEQGVCIRKNWNSSDYLHLNPDNFAIQLEKGGKFTVRGKPTLEDLEQFSEKFYCSCYSTLSCKEKADVKDTDAVDVCIADGVCIDAFLKPPMETEESQIFYNASPSTLSATMFIVSILFLIISSVASL

SEQ ID NO: 5 - protein, 509 aa, synthetic construct
  REGION 1..509: note = Synthetic Sequence
MGVLKFKHIFFRSFVKSSGVSQIVFTFLLIPCCLTLNFRAPPVIPNVPFLWAWNAPSKFCLGKFDEPLDMSLFSLIGSPRINITGQGVTIFYVDRLGYYPYIDSITGVTVNGGIPQKISLQDHLDKAKKDITFYMPVDNLGMAVIDWEEWRPTWARNWKPKDVYKNRSIELVQQQNVQLSLTEATEKAKQEFEKAGKDFMVETIKLGKLLRPNHLWGYYLFPDCYNHHYKKPGYNGSCFNVEIKRNDDLSWLWNESTALYPSIYLNTQQSPVAATLYVRNRVQEAIRVSKIPDAKSPLPVFVYTRIVFTDQVLKFLSQDELVYTFGETVALGASGIVIWGTLSIMRSMKSCLLLDNYMETILNPYIINVTLAAKMCSQVLCQEQGVCIRKDWNSSDYLHLNPDNFAIQLEKGGKFTVRGKPTLEDLEQFSEKFYCSCYSTLSCKEKADIKDTDAVDVCIADGVCIDAFLKPPMDTEESQIFYNASPSTLSATMLIVSILFLIISSVARL

SEQ ID NO: 6 - protein, 511 aa, synthetic construct
  REGION 1..511: note = Synthetic Sequence
MGVLKFKHIFFRSFVKSSGVSQIVLTFLLIPCCLTLNFRAPPIIPNMPFLWAWNAPSEFCLGKFDEPLDMSLFSLIGSPRINVTGQAVTIFYVDRLGYYPYIDSITGVTVNGGIPQKISLQDHLDKAKKDILFYMPVDNLGMAVIDWEEWRPTWARNWKPKDVYKNRSIELVQQQNVQLNLTEATEKAKQEFEKAGKDFMVETIKLGKLLRPNHLWGYYLFPDCYNHHYKKPGYNGSCFNVEIKRNDDLSWLWNESTALYPSIYLNTQQSPVAATLYVRNRVREAIRVSKIPDAKSPLPVFVYARIVFTDQVLKFLSQDELVYTFGETVALGASGIVIWGSLSIMRSMKSCLLLDNYMETILNPYIINVTLAAKMCSQVLCQEQGVCIRKDWNSSDYLHLNPDNFAIQLEKGGKFTVRGKPTLEDLEQFSEKFYCSCYSTLSCKEKADVKDTDAVDVCIADGVCIDAFLKPPMETEESQIFYNASPSTLSATMFIWRLEVWDQGISRMGFF

SEQ ID NO: 7 - protein, 509 aa, synthetic construct
  REGION 1..509: note = Synthetic Sequence
MGVLKFKHIFFRSFVKSNGVSQIVFTFLLIPRCLTLNFRAPPVIPNVPFLWAWNAPSEFCLGKFDEPLDMSLFSLIGSPRINVTGQGVTIFYVDRLGYYPYIDSITGVTVNGGIPQKISLQDHLDKAKQDITFYMPVDNLGMAVIDWEEWRPTWARNWKPKDVYKNRSIELVQQQNVQLNLTEATEKAKQEFEKAGKDFMVETIKLGKLLRPNHLWGYYLFPDCYNHHYKKPGYNGSCFNVEIKRNDDLSWLWNESTALYPSIYLNTQQSPVAATLYVRNRVREAIRVSKIPDAKSPLPVFVYARIVFTDQVLKFLSRDELVYTLGETVALGASGIVIWGSLSIMRSMKSCLLLDNYMETILNPYIINVTLAAKMCSQVLCQEQGVCIRKDWNSSDYLHLNPDNFAIQLEKGGKFTVRGKPTPEDLEQFSEKFYCSCYSTLSCKEKADVKDTDAVDVCIADGVCIDAFLKPPKETEESQIFYNASPSTLSATMFIVSILFPIISSVVSL

SEQ ID NO: 8 - protein, 509 aa, synthetic construct
  REGION 1..509: note = Synthetic Sequence
MGVLKFKHIFFRSFVKSNGISQIVFTFLLIPRCLTLNFRAPPVIPNVPFLWAWNAPSEFCLGKFDEPLDMSLFSLTGSPRINVTGQGVTIFYVDRLGYYPYIDSITGVTVNGGIPQKISLQDHLDKAKQDITFYMPVDNLGMAVIDWEEWRPTWARNWKPKDVYKNRSIELVQQQNVQLSLAEATEKAKQEFEKAGKDFMVETIKLGKLLRPNHLWGYYLFPDCYNHHYKKPGYNGSCFNVEIKRNDDLSWLWNESTALYPSIYLNTQQSPVAATLYVRNRVREAIRVSKIPDAKSPLPVFVYARIVFTDQVLKFLSRDELVYTLGETVALGASGIVIWGSLSIVRSMKSCLLLDNYMETILNPYIINVTLAAKMCSQVLCQEQGVCIRKDWNSSDYLHLNPDNFAIQLEKGGKFTVRGKPTPEDLEQFSEKFYCSCYSTLSCKEKADVKDTDAVDVCIADGVCIDAFLKPPKETEESQIFYNASPSTLSATMFIVSILFLIISSVVSL

SEQ ID NO: 9 - protein, 553 aa, synthetic construct
  REGION 1..553: note = Synthetic Sequence
MRMLRRHHISFRSFAGSSGTPQAVFTFLLLPCCLALDFRAPPLISNTSFLWAWNAPVERCVNRRFQLPPDLRLFSVKGSPQKSATGQFITLFYADRLGYYPHIDEKTGKTVFGGIPQLGNLKSHLEKAKNDIAYYIPNDSVGLAVIDWENWRPTWARNWKPKDVYRDESVELVLQKNPQLSFPEASKIAKVDFETAGKSFMQETLKLGKLLRPNHLWGYYLFPDCYNHNHNQPTYNGNCPDVEKRRNDDLEWLWKESTALFPSVYLNIRLKSTQNAALYVRNRVQEAIRLSKIASVESPLPVFVYARPVFTDGSSTYLSQGDLVNSVGEIVSLGASGIIMWGSLNLSLSMQSCMNLGTYLNTTLNPYIINVTLAAKMCSQVLCHNEGVCTRKHWNSSDYLHLNPMNFAIQTGEGGKYTVPGTVTLEDLQKFSDTFYCSCYANIHCKKRVDIKNVHSVNVCMAEDICIDSPVKLQPSDHSSSQEASTTTFSSISPSTTTATVSPCTPEKHSPECLKVRCSEVIPNVTQKACQSVKLKNISYQSPIQNIKNQTTY

SEQ ID NO: 10 - protein, 553 aa, synthetic construct
  REGION 1..553: note = Synthetic Sequence
KRMLRRRHISFRSFVGASGTPQAALAFLLLPCWLALDFRAPPLISNTSFLWAWNAPAERCVKIFKLPPDLRLFSVKGSPQKSATGQFITLFYADRLGYYPHIDEKTGNTVYGGIPQLGNLKNHLEKAKKDIAYYIPNDSVGLAVIDWENWRPTWARNWKPKDVYRDESVELVLQKNPQLSFPEASKIAKVDFETAGKSFMQETLKLGKLLRPNHLWGYYLFPDCYNHNYNQPTYNGNCSDLEKRRNDDLDWLWKESTALFPSVYLNIKLKSTPKAAFYVRNRVQEAIRLSKIASVESPLPVFVYHRPVFTDGSSTYLSQGDLVNSVGEIVALGASGIIMWGSLNLSLTMQSCMNLGNYLNTTLNPYIINVTLAAKMCSQVLCHDEGVCTRKQWNSSDYLHLNPMNFAIQTGKGGKYTVPGKVTLEDLQTFSDKFYCSCYANINCKKRVDIKNVHSVNVCMAEDICIEGPVKLQPSDHSSSQNEASTTTVSSISPSTTATTVSPCTPEKQSPECLKVRCLEAIANVTQTGCQGVKWKNTSSQSSIQNIKNQTTY